European Patent Specification EP 3 878 949 B1, published June 4, 2025. Title: REPROGRAMMING OF SOMATIC CELLS. Applicant: Whitehead Institute for Biomedical Research Jaenisch, Rudolf Hanna, Jacob Wernig, Marius Lengner, Christopher  J. Meissner, Alexander J. Brambrink, Oliver Tobias J. Welstead, G. Grant Foreman, Ruth. Application PCT/US2008/004516. The sequence listing filed with the application follows.

SEQUENCE LISTING (37 sequences)

SEQ ID NO: 1 - DNA, 22 bp, Artificial Sequence
  c-Myc forward primer
acctaactcgaggaggagctgg

SEQ ID NO: 2 - DNA, 21 bp, Artificial Sequence
  c-Myc reverse primer
tccacatagcgtaaaaggagc

SEQ ID NO: 3 - DNA, 20 bp, Artificial Sequence
  Klf4 forward primer
acactgtcttcccacgaggg

SEQ ID NO: 4 - DNA, 21 bp, Artificial Sequence
  Klf4 reverse primer
ggcattaaagcagcgtatcca

SEQ ID NO: 5 - DNA, 19 bp, Artificial Sequence
  Sox2 forward primer
cattaacggcacactgccc

SEQ ID NO: 6 - DNA, 21 bp, Artificial Sequence
  Sox2 reverse primer
ggcattaaagcagcgtatcca

SEQ ID NO: 7 - DNA, 21 bp, Artificial Sequence
  Oct4 forward primer
agcctggcctgtctgtcactc

SEQ ID NO: 8 - DNA, 21 bp, Artificial Sequence
  Oct4 reverse primer
ggcattaaagcagcgtatcca

SEQ ID NO: 9 - DNA, 20 bp, Artificial Sequence
  GAPDH forward primer
ttcaccaccatggagaaggc

SEQ ID NO: 10 - DNA, 18 bp, Artificial Sequence
  GAPDH reverse primer
cccttttggctccaccct

SEQ ID NO: 11 - RNA, 19 nt, Artificial Sequence
  Human Dnmt1-targeting siRNA
ggaagaagaguuacuauaa

SEQ ID NO: 12 - RNA, 19 nt, Artificial Sequence
  Human Dnmt1-targeting siRNA
gagcggaggugucccaaua

SEQ ID NO: 13 - RNA, 19 nt, Artificial Sequence
  Human Dnmt1-targeting siRNA
ggacgacccugaccucaaa

SEQ ID NO: 14 - RNA, 19 nt, Artificial Sequence
  Human Dnmt1-targeting siRNA
gaacggugcucaugcuuac

SEQ ID NO: 15 - RNA, 18 nt, Artificial Sequence
  Human Dnmt1-targeting siRNA
uuucucccucagacacuc

SEQ ID NO: 16 - RNA, 19 nt, Artificial Sequence
  Human Dnmt3a-targeting siRNA
gcacaaggguaccuacggg

SEQ ID NO: 17 - RNA, 19 nt, Artificial Sequence
  Human Dnmt3a-targeting siRNA
caagagagcggcuggugua

SEQ ID NO: 18 - RNA, 19 nt, Artificial Sequence
  Human Dnmt3a-targeting siRNA
gcacugaaauggaaagggu

SEQ ID NO: 19 - RNA, 19 nt, Artificial Sequence
  Human Dnmt3a-targeting siRNA
gaacugcuuucuggagugu

SEQ ID NO: 20 - RNA, 19 nt, Artificial Sequence
  Human Dnmt3b-targeting siRNA
gaaaguacgucgcuucuga

SEQ ID NO: 21 - RNA, 19 nt, Artificial Sequence
  Human Dnmt3b-targeting siRNA
acaaauggcuucagauguu

SEQ ID NO: 22 - RNA, 19 nt, Artificial Sequence
  Human Dnmt3b-targeting siRNA
gcucuuaccuuaccaucga

SEQ ID NO: 23 - RNA, 19 nt, Artificial Sequence
  Human Dnmt3b-targeting siRNA
uuuaccaccugcugaauua

SEQ ID NO: 24 - RNA, 21 nt, Artificial Sequence
  Human Hprt-targeting siRNA
ccaguuucacuaaugacacaa

SEQ ID NO: 25 - RNA, 19 nt, Artificial Sequence
  Mouse Dnmt1-targeting siRNA
ggaaagagauggcuuaaca

SEQ ID NO: 26 - RNA, 19 nt, Artificial Sequence
  Mouse Dnmt1-targeting siRNA
gcugggagauggcgucaua

SEQ ID NO: 27 - RNA, 19 nt, Artificial Sequence
  Mouse Dnmt1-targeting siRNA
gauaagaaacgcagaguug

SEQ ID NO: 28 - RNA, 19 nt, Artificial Sequence
  Mouse Dnmt1-targeting siRNA
gguagagaguuacgacgaa

SEQ ID NO: 29 - RNA, 19 nt, Artificial Sequence
  Mouse Dnmt3a-targeting siRNA
cgcgauuucuugagucuaa

SEQ ID NO: 30 - RNA, 19 nt, Artificial Sequence
  Mouse Dnmt3a-targeting siRNA
cgaauugugucuuggugga

SEQ ID NO: 31 - RNA, 19 nt, Artificial Sequence
  Mouse Dnmt3a-targeting siRNA
aaacaucgaggacauuugu

SEQ ID NO: 32 - RNA, 19 nt, Artificial Sequence
  Mouse Dnmt3a-targeting siRNA
caagggacuuuaugagggu

SEQ ID NO: 33 - RNA, 19 nt, Artificial Sequence
  Mouse Dnmt3b-targeting siRNA
gcaaugaucucucuaacgu

SEQ ID NO: 34 - RNA, 19 nt, Artificial Sequence
  Mouse Dnmt3b-targeting siRNA
ggaaugcgcuggguacagu

SEQ ID NO: 35 - RNA, 19 nt, Artificial Sequence
  Mouse Dnmt3b-targeting siRNA
uaaucuggcuaccuucaau

SEQ ID NO: 36 - RNA, 19 nt, Artificial Sequence
  Mouse Dnmt3b-targeting siRNA
gcaaagguuuauaugaggg

SEQ ID NO: 37 - RNA, 21 nt, Artificial Sequence
  Mouse Hprt-targeting siRNA
ccaguuucacuaaugacacaa